European Patent Application EP 4 628 590 A1, published October 8, 2025. Title: A microorganism expressing threonine export protein RhtC and a use for producing L-isoleucine thereof. Applicant: CJ CheilJedang Corporation. The sequence listing filed with the application follows.

SEQUENCE LISTING (16 sequences)

SEQ ID NO: 1 - DNA, 40 bp, synthetic construct
  misc_feature 1..40: note = Primer1
  source 1..40: mol_type = other DNA
tgaattcgagctcggtaccctcatattgaatttcgcccca

SEQ ID NO: 2 - DNA, 40 bp, synthetic construct
  misc_feature 1..40: note = Primer2
  source 1..40: mol_type = other DNA
cctaagcaggttgatttagtactccgctggaaaacatttt

SEQ ID NO: 3 - DNA, 40 bp, synthetic construct
  misc_feature 1..40: note = Primer3
  source 1..40: mol_type = other DNA
aaaatgttttccagcggagtactaaatcaacctgcttagg

SEQ ID NO: 4 - DNA, 40 bp, synthetic construct
  misc_feature 1..40: note = Primer4
  source 1..40: mol_type = other DNA
gtcgactctagaggatcccctcccaccaaatctgcgccca

SEQ ID NO: 5 - DNA, 40 bp, synthetic construct
  misc_feature 1..40: note = Primer5
  source 1..40: mol_type = other DNA
aaaatgttttccagcggagtattcagggtagttgactaaa

SEQ ID NO: 6 - DNA, 34 bp, synthetic construct
  misc_feature 1..34: note = Primer6
  source 1..34: mol_type = other DNA
aataacatcaacatctttgtgcacctttcgatct

SEQ ID NO: 7 - DNA, 40 bp, synthetic construct
  misc_feature 1..40: note = Primer7
  source 1..40: mol_type = other DNA
agatcgaaaggtgcacaaagatgttgatgttatttctcac

SEQ ID NO: 8 - DNA, 30 bp, synthetic construct
  misc_feature 1..30: note = Primer8
  source 1..30: mol_type = other DNA
attttttcgataatcgaatgcaggccaagc

SEQ ID NO: 9 - DNA, 30 bp, synthetic construct
  misc_feature 1..30: note = Primer9
  source 1..30: mol_type = other DNA
gcttggcctgcattcgattatcgaaaaaat

SEQ ID NO: 10 - DNA, 40 bp, synthetic construct
  misc_feature 1..40: note = Primer10
  source 1..40: mol_type = other DNA
cctaagcaggttgatttagttcaccgcgaaataatcaaat

SEQ ID NO: 11 - protein, 206 aa, synthetic construct
  REGION 1..206: note = rhtC wild-type
MLMLFLTVAMVHIVALMSPGPDFFFVSQTAVSRSRKEAMMGVLGITCGVMVWAGIALLGLHLIIEKMAWLHTLIMVGGGLYLCWMGYQMLRGALKKEAVSAPAPQVELAKSGRSFLKGLLTNLANPKAIIYFGSVFSLFVGDNVGTTARWGIFALIIVETLAWFTVVASLFALPQMRRGYQRLAKWIDGFAGALFAGFGIHLIISR

SEQ ID NO: 12 - DNA, 621 bp, synthetic construct
  misc_feature 1..621: note = rhtC wild-type coding DNA
  source 1..621: mol_type = other DNA
atgttgatgttatttctcaccgtcgccatggtgcacattgtggcgcttatgagccccggtcccgatttcttttttgtctctcagaccgctgtcagtcgttcccgtaaagaagcgatgatgggcgtgctgggcattacctgcggcgtaatggtttgggctgggattgcgctgcttggcctgcatttgattatcgaaaaaatggcctggctgcatacgctgattatggtgggcggtggcctgtatctctgctggatgggttaccagatgctacgtggtgcactgaaaaaagaggcggtttctgcacctgcgccacaggtcgagctggcgaaaagtgggcgcagtttcctgaaaggtttactgaccaatctcgctaatccgaaagcgattatctactttggctcggtgttctcattgtttgtcggtgataacgttggcactaccgcgcgctggggcatttttgcgctgatcattgtcgaaacgctggcgtggtttaccgtcgttgccagcctgtttgccctgccgcaaatgcgccgtggttatcaacgtctggcgaagtggattgatggttttgccggggcgttatttgccggatttggcattcatttgattatttcgcggtga

SEQ ID NO: 13 - protein, 206 aa, synthetic construct
  REGION 1..206: note = rhtC L62S
MLMLFLTVAMVHIVALMSPGPDFFFVSQTAVSRSRKEAMMGVLGITCGVMVWAGIALLGLHSIIEKMAWLHTLIMVGGGLYLCWMGYQMLRGALKKEAVSAPAPQVELAKSGRSFLKGLLTNLANPKAIIYFGSVFSLFVGDNVGTTARWGIFALIIVETLAWFTVVASLFALPQMRRGYQRLAKWIDGFAGALFAGFGIHLIISR

SEQ ID NO: 14 - DNA, 621 bp, synthetic construct
  misc_feature 1..621: note = rhtC L62S coding DNA
  source 1..621: mol_type = other DNA
atgttgatgttatttctcaccgtcgccatggtgcacattgtggcgcttatgagccccggtcccgatttcttttttgtctctcagaccgctgtcagtcgttcccgtaaagaagcgatgatgggcgtgctgggcattacctgcggcgtaatggtttgggctgggattgcgctgcttggcctgcattcgattatcgaaaaaatggcctggctgcatacgctgattatggtgggcggtggcctgtatctctgctggatgggttaccagatgctacgtggtgcactgaaaaaagaggcggtttctgcacctgcgccacaggtcgagctggcgaaaagtgggcgcagtttcctgaaaggtttactgaccaatctcgctaatccgaaagcgattatctactttggctcggtgttctcattgtttgtcggtgataacgttggcactaccgcgcgctggggcatttttgcgctgatcattgtcgaaacgctggcgtggtttaccgtcgttgccagcctgtttgccctgccgcaaatgcgccgtggttatcaacgtctggcgaagtggattgatggttttgccggggcgttatttgccggatttggcattcatttgattatttcgcggtga

SEQ ID NO: 15 - DNA, 611 bp, synthetic construct
  misc_feature 1..611: note = PlysCP1
  source 1..611: mol_type = other DNA
ccatcttttggggtgcggagcgcgatccggtgtctgaccacggtgccccatgcgattgttaatgccgatgctagggcgaaaagcacggcgagcagattgctttgcacttgattcagggtagttgactaaagagttgctcgcgaagtagcacctgtcacttttgtctcaaatattaaatcgaatatcaatatatggtctgtttattggaacgcgtcccagtggctgagacgcatccgctaaagccccaggaaccctgtgcagaaagaaaacactcctctggctaggtagacacagtttattgtggtagagttgagcgggtaactgtcagcacgtagatcgaaaggtgcacaaaggtggccctggtcgtacagaaatatggcggttcctcgcttgagagtgcggaacgcattagaaacgtcgctgaacggatcgttgccaccaagaaggctggaaatgatgtcgtggttgtctgctccgcaatgggagacaccacggatgaacttctagaacttgcagcggcagtgaatcccgttccgccagctcgtgaaatggatatgctcctgactgctggtgagcgtatttctaacgctctcgtcgccatggctattgag

SEQ ID NO: 16 - DNA, 5802 bp, synthetic construct
  source 1..5802: mol_type = other DNA
  misc_feature 1..5802: note = pDC24 vector
gttcgcttgctgtccataaaaccgcccagtctagctatcgccatgtaagcccactgcaagctacctgctttctctttgcgcttgcgttttcccttgtccagatagcccagtagctgacattcatccggggtcagcaccgtttctgcggactggctttctacgtgttccgcttcctttagcagcccttgcgccctgagtgcttgcggcagcgtgaagctagcttttatcgccattcgccattcaggctgcgcaactgttgggaagggcgatcggtgcgggcctcttcgctattacgccagctggcgaaagggggatgtgctgcaaggcgattaagttgggtaacgccagggttttcccagtcacgacgttgtaaaacgacggccagtgaattcgagctcggtacccggggatcctctagagtcgacctgcaggcatgcaagcttggcgtaatcatggtcatagctgtttcctgtgtgaaattgttatccgctcacaattccacacaacatacgagccggaagcataaagtgtaaagcctggggtgcctaatgagtgagctaactcacattaattgcgttgcgctcactgcccgctttccagtcgggaaacctgtcgtgccagctgcattaatgaatcggccaacgcgcggggagaggcggtttgcgtattgggcgctcttccgcttcctcgctcactgactcgctgcgctcggtcgttcggctgcggcgagcggtatcagctcactcaaaggcggtaatacggttatccacagaatcaggggataacgcaggaaagaacatgtgagcaaaaggccagcaaaaggccaggaaccgtaaaaaggccgcgttgctggcgtttttccataggctccgcccccctgacgagcatcacaaaaatcgacgctcaagtcagaggtggcgaaacccgacaggactataaagataccaggcgtttccccctggaagctccctcgtgcgctctcctgttccgaccctgccgcttaccggatacctgtccgcctttctcccttcgggaagcgtggcgctttctcaatgctcacgctgtaggtatctcagttcggtgtaggtcgttcgctccaagctgggctgtgtgcacgaaccccccgttcagcccgaccgctgcgccttatccggtaactatcgtcttgagtccaacccggtaagacacgacttatcgccactggcagcagccactggtaacaggattagcagagcgaggtatgtaggcggtgctacagagttcttgaagtggtggcctaactacggctacactagaaggacagtatttggtatctgcgctctgctgaagccagttaccttcggaaaaagagttggtagctcttgatccggcaaacaaaccaccgctggtagcggtggtttttttgtttgcaagcagcagattacgcgcagaaaaaaaggatctcaagaagatcctttgatcttttctacggggtctgacgctcagtggaacgaaaactcacgttaagggattttggtcatgagattatcaaaaaggatcttcacctagatccttttggggtgggcgaagaactccagcatgagatccccgcgctggaggatcatccagccctgatagaaacagaagccactggagcacctcaaaaacaccatcatacactaaatcagtaagttggcagcatcacccgacgcactttgcgccgaataaatacctgtgacggaagatcacttcgcagaataaataaatcctggtgtccctgttgataccgggaagccctgggccaacttttggcgaaaatgagacgttgatcggcacgtaagaggttccaactttcaccataatgaaataagatcactaccgggcgtattttttgagttatcgagattttcaggagctgatagaaacagaagccactggagcacctcaaaaacaccatcatacactaaatcagtaagttggcagcatcacccgacgcactttgcgccgaataaatacctgtgacggaagatcacttcgcagaataaataaatcctggtgtccctgttgataccgggaagccctgggccaacttttggcgaaaatgagacgttgatcggcacgtaagaggttccaactttcaccataatgaaataagatcactaccgggcgtattttttgagttatcgagattttcaggagctctttggcatcgtctctcgcctgtcccctcagttcagtaatttcctgcatttgcctgtttccagtcggtagatattccacaaaacagcagggaagcagcgcttttccgctgcataaccctgcttcggggtcattatagcgattttttcggtatatccatcctttttcgcacgatatacaggattttgccaaagggttcgtgtagactttccttggtgtatccaacggcgtcagccgggcaggataggtgaagtaggcccacccgcgagcgggtgttccttcttcactgtcccttattcgcacctggcggtgctcaacgggaatcctgctctgcgaggctggccggctaccgccggcgtaacagatgagggcaagcggatggctgatgaaaccaagccaaccaggaagggcagcccacctatcaaggtgtactgccttccagacgaacgaagagcgattgaggaaaaggcggcggcggccggcatgagcctgtcggcctacctgctggccgtcggccagggctacaaaatcacgggcgtcgtggactatgagcacgtccgcgagggcgtcccggaaaacgattccgaagcccaacctttcatagaaggcggcggtggaatcgaaatctcgtgatggcaggttgggcgtcgcttggtcggtcatttcgaaaaaggttaggaatacggttagccatttgcctgcttttatatagttcatatgggattcacctttatgttgataagaaataaaagaaaatgccaataggatatcggcattttcttttgcgtttttatttgttaactgttaattgtccttgttcaaggatgctgtctttgacaacagatgttttcttgcctttgatgttcagcaggaagctcggcgcaaacgttgattgtttgtctgcgtagaatcctctgtttgtcatatagcttgtaatcacgacattgtttcctttcgcttgaggtacagcgaagtgtgagtaagtaaaggttacatcgttaggcggatcaagatccatttttaacacaaggccagttttgttcagcggcttgtatgggccagttaaagaattagaaacataaccaagcatgtaaatatcgttagacgtaatgccgtcaatcgtcatttttgatccgcgggagtcagtgaacaggtaccatttgccgttcattttaaagacgttcgcgcgttcaatttcatctgttactgtgttagatgcaatcagcggtttcatcacttttttcagtgtgtaatcatcgtttagctcaatcataccgagagcgccgtttgctaactcagccgtgcgttttttatcgctttgcagaagtttttgactttcttgacggaagaatgatgtgcttttgccatagtatgctttgttaaataaagattcttcgccttggtagccatcttcagttccagtgtttgcttcaaatactaagtatttgtggcctttatcttctacgtagtgaggatctctcagcgtatggttgtcgcctgagctgtagttgccttcatcgatgaactgctgtacattttgatacgtttttccgtcaccgtcaaagattgatttataatcctctacaccgttgatgttcaaagagctgtctgatgctgatacgttaacttgtgcagttgtcagtgtttgtttgccgtaatgtttaccggagaaatcagtgtagaataaacggatttttccgtcagatgtaaatgtggctgaacctgaccattcttgtgtttggtcttttaggatagaatcatttgcatcgaatttgtcgctgtctttaaagacgcggccagcgtttttccagctgtcaatagaagtttcgccgactttttgatagaacatgtaaatcgatgtgtcatccgcatttttaggatctccggctaatgcaaagacgatgtggtagccgtgatagtttgcgacagtgccgtcagcgttttgtaatggccagctgtcccaaacgtccaggccttttgcagaagagatatttttaattgtggacgaatcaaattcagaaacttgatatttttcatttttttgctgttcagggatttgcagcatatcatggcgtgtaatatgggaaatgccgtatgtttccttatatggcttttggttcgtttctttcgcaaacgcttgagttgcgcctcctgccagcagtgcggtagtaaaggttaatactgttgcttgttttgcaaactttttgatgttcatcgttcatgtctccttttttatgtactgtgttagcggtctgcttcttccagccctcctgtttgaagatggcaagttagttacgcacaataaaaaaagacctaaaatatgtaaggggtgacgccaaagtatacactttgccctttacacattttaggtcttgcctgctttatcagtaacaaacccgcgcgatttacttttcgacctcattctattagactctcgtttggattgcaactggtctattttcctcttttgtttgatagaaaatcataaaaggatttgcagactacgggcctaaagaactaaaaaatctatctgtttcttttcattctctgtattttttatagtttctgttgcatgggcataaagttgcctttttaatcacaattcagaaaatatcataatatctcatttcactaaataatagtgaacggcaggtatatgtgatgggttaaaaaggatcaccccagagtcccgctcagaagaactcgtcaagaaggcgatagaaggcgatgcgctgcgaatcgggagcggcgataccgtaaagcacgaggaagcggtcagcccattcgccgccaagctcttcagcaatatcacgggtagccaacgctatgtcctgatagcggtccgccacacccagccggccacagtcgatgaatccagaaaagcggccattttccaccatgatattcggcaagcaggcatcgccatgggtcacgacgagatcctcgccgtcgggcatccgcgccttgagcctggcgaacagttcggctggcgcgagcccctgatgctcttcgtccagatcatcctgatcgacaagaccggcttccatccgagtacgtgctcgctcgatgcgatgtttcgcttggtggtcgaatgggcaggtagccggatcaagcgtatgcagccgccgcattgcatcagccatgatggatactttctcggcaggagcaaggtgagatgacaggagatcctgccccggcacttcgcccaatagcagccagtcccttcccgcttcagtgacaacgtcgagacagctgcgcaaggaacgcccgtcgtggccagccacgatagccgcgctgcctcgtcttggagttcattcagggcaccggacaggtcggtcttgacaaaaagaaccgggcgcccctgcgctgacagccggaacacggcggcatcagagcagccgattgtctgttgtgcccagtcatagccgaatagcctctccacccaagcggccggagaacctgcgtgcaatccatcttgttcaatcatgcgaaacgatcctcatcctgtctcttgatcagatcttgatcccctgcgccatcagatccttggcggcaagaaagccatccagtttactttgcagggcttcccaaccttaccagagggcgccccagctggcaattccg